European Patent Specification EP 3 618 834 B1, published June 26, 2024. Title: Functionalized saccharides as anti-inflammatory agents. Applicant: HuVePharma. The sequence listing filed with the application follows.

SEQUENCE LISTING (14 sequences)

SEQ ID NO: 1 - DNA, 23 bp, Artificial Sequence
  Synthesized Oligonucleotide
aaaacamaggcgatcgccctgta

SEQ ID NO: 2 - DNA, 22 bp, Artificial Sequence
  Synthesized Oligonucleotide
tttcttcgccaggttcaaagcg

SEQ ID NO: 3 - DNA, 20 bp, Artificial Sequence
  Synthesized Oligonucleotide
ctgacctagagaagacacat

SEQ ID NO: 4 - DNA, 20 bp, Artificial Sequence
  Synthesized Oligonucleotide
ggtcagtgaagtaaaggtac

SEQ ID NO: 5 - DNA, 22 bp, Artificial Sequence
  Synthesized Oligonucleotide
cacctcacaagcagagcacaag

SEQ ID NO: 6 - DNA, 25 bp, Artificial Sequence
  Synthesized Oligonucleotide
gcattagaaacagtccagcccatac

SEQ ID NO: 7 - DNA, 21 bp, Artificial Sequence
  Synthesized Oligonucleotide
tgcctgaagaccctgccaagg

SEQ ID NO: 8 - DNA, 21 bp, Artificial Sequence
  Synthesized Oligonucleotide
gttagccttgcctttgttcag

SEQ ID NO: 9 - DNA, 20 bp, Artificial Sequence
  Synthesized Oligonucleotide
ggtatcacccctcgtcactt

SEQ ID NO: 10 - DNA, 20 bp, Artificial Sequence
  Synthesized Oligonucleotide
tcagcgatttgtggatgtgt

SEQ ID NO: 11 - DNA, 20 bp, Artificial Sequence
  Synthesized Oligonucleotide
caggccagactttgttggat

SEQ ID NO: 12 - DNA, 20 bp, Artificial Sequence
  Synthesized Oligonucleotide
ttgcgctcatcttaggcttt

SEQ ID NO: 13 - DNA, 20 bp, Artificial Sequence
  Synthesized Oligonucleotide
agcatacaggtcctggcatc

SEQ ID NO: 14 - DNA, 20 bp, Artificial Sequence
  Synthesized Oligonucleotide
ttcaccttcccaaagaccac